European Patent Specification EP 3 719 499 B1, published February 22, 2023. Title: Method and reagent for measuring hepatitis B virus s antigen. Applicant: FUJIREBIO, INC. The sequence listing filed with the application follows.

SEQUENCE LISTING (1 sequence)

SEQ ID NO: 1 - protein, 226 aa, Hepatitis B virus
MENITSGFLGPLLVLQAGFFLLTRILTIPQSLDSWWTSLNFLGGSPVCLGQNSQSPTSNHSPTSCPPICPGYRWMCLRRFIIFLFILLLCLIFLIVLLDYQGMLPVCPLIPGSTTTSTGPCKTCTTPAQGNSMFPSCCCTKPTDGNCTCIPIPSSWAFAKYLWEWASVRFSWLSLLVPFVQWFVGLSPTVWLSAIWMMWYWGPSLYSIVSPFLPLLPIFFCLWVYI